European Patent Specification EP 4 277 747 B1, published March 19, 2025. Title: ANALYSIS OF CELLS AND/OR ORGANELLES IN HYDROGEL CAGES. Applicant: PARIS SCIENCES ET LETTRES - QUARTIER LATIN ECOLE SUPERIEURE DE PHYSIQUE ET DE CHIMIE INDUSTRIELLES DE LA VILLE DE PARIS CENTRE NATIONALE DE LA RECHERCHE SCIENTIFIQUE MICROFACTORY SAS. The sequence listing filed with the application follows.

SEQUENCE LISTING (21 sequences)

SEQ ID NO: 1 - DNA, 25 bp, Artificial Sequence
  Oligonucleotide
tgctagctcgccaccgcagccacaa

SEQ ID NO: 2 - DNA, 64 bp, Artificial Sequence
  Oligonucleotide
  misc_feature (21)..(32): n is a, c, g, or t
  misc_feature (64)..(64): n is a, c, g, or t
ccactctagccgttcggaacnnnnnnnnnnnnttttttttttttttttttttttttttttttvn

SEQ ID NO: 3 - DNA, 15 bp, Artificial Sequence
  Oligonucleotide
acatgcgttctctgg

SEQ ID NO: 4 - DNA, 15 bp, Artificial Sequence
  Oligonucleotide
tggaaggttgagcga

SEQ ID NO: 5 - DNA, 15 bp, Artificial Sequence
  Oligonucleotide
ccgaacaaccagact

SEQ ID NO: 6 - DNA, 29 bp, Artificial Sequence
  Oligonucleotide
caagcagaagacggcatacgagatrgrgg

SEQ ID NO: 7 - DNA, 79 bp, Artificial Sequence
  Oligonucleotide
  misc_feature (59)..(64): n is a, c, g, or t
aatgatacggcgaccaccgagatctacactctttccctacacgacgctcttccgatctnnnnnnctagcgcgcagtgac

SEQ ID NO: 8 - DNA, 24 bp, Artificial Sequence
  Oligonucleotide
caagcagaagacggcatacgagat

SEQ ID NO: 9 - DNA, 30 bp, Artificial Sequence
  Oligonucleotide
gtgtagggaaagagtgtgctagcgcacaat

SEQ ID NO: 10 - DNA, 58 bp, Artificial Sequence
  Oligonucleotide
aatgatacggcgaccaccgagatctacactctttccctacacgacgctcttccgatct

SEQ ID NO: 11 - DNA, 52 bp, Artificial Sequence
  Oligonucleotide
  misc_feature (21)..(32): n is a, c, g, or t
ccactctagccgttcggaacnnnnnnnnnnnngcaatttgtgagggccgttc

SEQ ID NO: 12 - DNA, 49 bp, Artificial Sequence
  Oligonucleotide
caagcagaagacggcatacgagatccttaccactcggccatgccgccaa

SEQ ID NO: 13 - DNA, 26 bp, Artificial Sequence
  Oligonucleotide
ctcacgcgcagacacgcgttgcgctg

SEQ ID NO: 14 - DNA, 57 bp, Artificial Sequence
  Oligonucleotide
  misc_feature (14)..(25): n is a, c, g, or t
  misc_feature (57)..(57): n is a, c, g, or t
gtctgcgcgtgagnnnnnnnnnnnnttttttttttttttttttttttttttttttvn

SEQ ID NO: 15 - DNA, 79 bp, Artificial Sequence; identical to SEQ ID NO: 7
  Oligonucleotide
  misc_feature (59)..(64): n is a, c, g, or t

SEQ ID NO: 16 - DNA, 47 bp, Artificial Sequence
  Oligonucleotide
caagcagaagacggcatacgagatttgtggctgcggtggcgagctag

SEQ ID NO: 17 - DNA, 60 bp, Artificial Sequence
  Oligonucleotide
gttccgaacggctagagtggtcgctcaaccttccattgtggctgcggtggcgagctagca

SEQ ID NO: 18 - DNA, 105 bp, Artificial Sequence
  Oligonucleotide
  misc_feature (62)..(73): n is a, c, g, or t
  misc_feature (105)..(105): n is a, c, g, or t
attgtgcgctagcacactctttccctacacgacgctcttccgatcttcgctcaaccttccannnnnnnnnnnnttttttttttttttttttttttttttttttvn

SEQ ID NO: 19 - DNA, 81 bp, Artificial Sequence
  Oligonucleotide
caatcactgtgaccgccctgaatgatcaccttaccactcggccatgccgccaacacaacacgaacggccctcacaaattgc

SEQ ID NO: 20 - DNA, 60 bp, Artificial Sequence
  Oligonucleotide
cgctagcgcgcagtgactcgctcaaccttccacagcgcaacgcgtcactgcgcgctagcg

SEQ ID NO: 21 - DNA, 60 bp, Artificial Sequence
  Oligonucleotide
ctgtctcttatacacatcttcgctcaaccttccattgtggctgcggtggcgagctagcag